European Patent Specification EP 3 368 085 B1, published January 3, 2024. Title: Modified Alginates for Anti-Fibrotic Materials and Applications. Applicant: Massachusetts Institute of Technology The Children's Medical Center Corporation Vegas, Arturo J. Doloff, Joshua C. Veiseh, Omid Ma, Minglin Langer, Robert S. Anderson, Daniel G. The sequence listing filed with the application follows.

SEQUENCE LISTING (24 sequences)

SEQ ID NO: 1 - DNA, 21 bp, Artificial Sequence
  Synthetic Primer
catgttcagctttgtggacct

SEQ ID NO: 2 - DNA, 20 bp, Artificial Sequence
  Synthetic Primer
gcagctgacttcagggatgt

SEQ ID NO: 3 - DNA, 22 bp, Artificial Sequence
  Synthetic Primer
gcaggttcacctactctgtcct

SEQ ID NO: 4 - DNA, 20 bp, Artificial Sequence
  Synthetic Primer
cttgccccattcatttgtct

SEQ ID NO: 5 - DNA, 21 bp, Artificial Sequence
  Synthetic Primer
cgcttccgctgcccagagact

SEQ ID NO: 6 - DNA, 26 bp, Artificial Sequence
  Synthetic Primer
tataggtggtttcgtggatgcccgct

SEQ ID NO: 7 - DNA, 22 bp, Artificial Sequence
  Synthetic Primer
ccaagagaatgcaaaaggcttt

SEQ ID NO: 8 - DNA, 20 bp, Artificial Sequence
  Synthetic Primer
ggggggctgcaacaaccaca

SEQ ID NO: 9 - DNA, 21 bp, Artificial Sequence
  Synthetic Primer
gcccgagtacagtctacctgg

SEQ ID NO: 10 - DNA, 20 bp, Artificial Sequence
  Synthetic Primer
agagatgaattctgcgccat

SEQ ID NO: 11 - DNA, 20 bp, Artificial Sequence
  Synthetic Primer
tgccccttctctgatggatt

SEQ ID NO: 12 - DNA, 22 bp, Artificial Sequence
  Synthetic Primer
tgctcttgacttgcttctgtga

SEQ ID NO: 13 - DNA, 22 bp, Artificial Sequence
  Synthetic Primer
gcttctttgcagctccttcgtt

SEQ ID NO: 14 - DNA, 20 bp, Artificial Sequence
  Synthetic Primer
cggagccgttctcgacgacc

SEQ ID NO: 15 - DNA, 21 bp, Artificial Sequence
  Synthetic Primer
catgttcagctttgtggacct

SEQ ID NO: 16 - DNA, 20 bp, Artificial Sequence
  Synthetic Primer
gcagctgacttcagggatgt

SEQ ID NO: 17 - DNA, 19 bp, Artificial Sequence
  Synthetic Primer
cctggctctcgaggtgaac

SEQ ID NO: 18 - DNA, 18 bp, Artificial Sequence
  Synthetic Primer
caatgcccagaggaccag

SEQ ID NO: 19 - DNA, 21 bp, Artificial Sequence
  Synthetic Primer
tgccatgtatgtggctattca

SEQ ID NO: 20 - DNA, 21 bp, Artificial Sequence
  Synthetic Primer
accagttgtacgtccagaagc

SEQ ID NO: 21 - DNA, 19 bp, Artificial Sequence
  Synthetic Primer
ctctcgtgccatgtgaacc

SEQ ID NO: 22 - DNA, 22 bp, Artificial Sequence
  Synthetic Primer
ttctctaaattggtcccaggaa

SEQ ID NO: 23 - DNA, 22 bp, Artificial Sequence
  Synthetic Primer
accttcttgcagctcctccgtc

SEQ ID NO: 24 - DNA, 20 bp, Artificial Sequence
  Synthetic Primer
cggagccgttgtcgacgacg